European Patent Specification EP 3 342 783 B1, published December 4, 2024. Title: Method for controlling affinity of antibody for antigen, antibody whose affinity for antigen has been altered, and its production method. Applicant: SYSMEX CORPORATION. The sequence listing filed with the application follows.

SEQUENCE LISTING (25 sequences)

SEQ ID NO: 1 - DNA, 40 bp, Artificial Sequence
  primer
ttcgtattcggtcccttccccttcgccttcaaagcgagca

SEQ ID NO: 2 - DNA, 40 bp, Artificial Sequence
  primer
atcgtaatcggtcccatccccatcgccatcaaagcgagca

SEQ ID NO: 3 - DNA, 40 bp, Artificial Sequence
  primer
cttgtacttggtccccttccccttgcccttaaagcgagca

SEQ ID NO: 4 - DNA, 40 bp, Artificial Sequence
  primer
tctgtatctggtccctctccctctgcctctaaagcgagca

SEQ ID NO: 5 - DNA, 18 bp, Artificial Sequence
  primer
ctcacaatcagctgattg

SEQ ID NO: 6 - DNA, 25 bp, Artificial Sequence
  primer
tctccctctgcctctaaagcgagca

SEQ ID NO: 7 - DNA, 15 bp, Artificial Sequence
  primer
gggaccagatacaga

SEQ ID NO: 8 - DNA, 25 bp, Artificial Sequence
  primer
ggcacagacgccgacctggcaatca

SEQ ID NO: 9 - DNA, 25 bp, Artificial Sequence
  primer
gtcccggtctccgtcaaaccggtcg

SEQ ID NO: 10 - DNA, 25 bp, Artificial Sequence
  primer
ggcacagaggccgagctggcaatca

SEQ ID NO: 11 - DNA, 25 bp, Artificial Sequence
  primer
ctcccgctctccctcaaaccggtcg

SEQ ID NO: 12 - DNA, 25 bp, Artificial Sequence
  primer
ggcacaaaggccaagctggcaatca

SEQ ID NO: 13 - DNA, 25 bp, Artificial Sequence
  primer
cttccgctttcccttaaaccggtcg

SEQ ID NO: 14 - DNA, 25 bp, Artificial Sequence
  primer
ggcacaagggccaggctggcaatca

SEQ ID NO: 15 - DNA, 25 bp, Artificial Sequence
  primer
cctccgccttcccctaaaccggtcg

SEQ ID NO: 16 - protein, 10 aa, Homo sapiens
GNSSNIGNNA

SEQ ID NO: 17 - protein, 8 aa, Homo sapiens
WDDSLDSQ

SEQ ID NO: 18 - protein, 11 aa, Mus musculus
RASQSIGNNLH

SEQ ID NO: 19 - protein, 7 aa, Mus musculus
YASQSIS

SEQ ID NO: 20 - protein, 9 aa, Mus musculus
QQSNSWPYT

SEQ ID NO: 21 - protein, 5 aa, Mus musculus
SDYWS

SEQ ID NO: 22 - protein, 16 aa, Mus musculus
YVSYSGSTYYNPSLKS

SEQ ID NO: 23 - protein, 5 aa, Mus musculus
WDGDY

SEQ ID NO: 24 - DNA, 36 bp, Artificial Sequence
  primer
gggaccgattatgatctcacaatcagtcgaatggag

SEQ ID NO: 25 - DNA, 39 bp, Artificial Sequence
  primer
atccccatcggcatcgaaacgaacagggactccagaagc